European Patent Specification EP 3 572 516 B1, published November 20, 2024. Title: METHODS AND MATERIALS FOR ACTIVATING AN INTERNAL RIBOSOMAL ENTRY SITE IN EXON 5 OF THE DMD GENE. Applicant: Flanigan, et al. The sequence listing filed with the application follows.

SEQUENCE LISTING (34 sequences)

SEQ ID NO: 1 - DNA, 28 bp, Homo sapiens
tcaaaagaaaacattcacaaaatgggta

SEQ ID NO: 2 - DNA, 23 bp, Homo sapiens
gcacaattttctaaggtaagaat

SEQ ID NO: 3 - DNA, 31 bp, Homo sapiens
tagatgaaagagaagatgttcaaaagaaaac

SEQ ID NO: 4 - DNA, 21 bp, Homo sapiens
tagatgaaagagaagatgttc

SEQ ID NO: 5 - DNA, 28 bp, Adeno-associated virus
tacccattttgcgaatgttttcttttga

SEQ ID NO: 6 - DNA, 23 bp, Adeno-associated virus
attcttaccttagaaaattgtgc

SEQ ID NO: 7 - DNA, 31 bp, Adeno-associated virus
gttttcttttgaagatcttctctttcatcta

SEQ ID NO: 8 - DNA, 21 bp, Adeno-associated virus
gaagatcttctctttcatcta

SEQ ID NO: 9 - RNA, 28 nt, Homo sapiens
uacccauuuugcgaauguuuucuuuuga

SEQ ID NO: 10 - RNA, 23 nt, Homo sapiens
auucuuaccuuagaaaauugugc

SEQ ID NO: 11 - RNA, 31 nt, Homo sapiens
guuuucuuuugaacaucuucucuuucaucua

SEQ ID NO: 12 - RNA, 21 nt, Homo sapiens
gaacaucuucucuuucaucua

SEQ ID NO: 13 - RNA, 30 nt, Homo sapiens
ccauuuugugaauguuuucuuuugaacauc

SEQ ID NO: 14 - DNA, 4472 bp, Adeno-associated virus rh74
ctccatcactaggggtaaccgcgaagcgcctcccacgctgccgcgtcagcgctgacgtaaattacgtcataggggagtggtcctgtattagctgtcacgtgagtgcttttgcgacattttgcgacaccacgtggccattcatggtatatatggccgagtgagcgagcaggatctccattttgaccgcgaaatttgaacgagcagcagccatgccgggcttctacgagatcgtgcttaaggtgccgagcgacctggacgagcacctgccgggcatttctgactcgtttgtgaactgggtggcagagaaggaatgggagctgcccccggattctgacatggatcggaatctgattgagcaggcacccctgaccgtggccgagaagctacagcgcgacttcctggtccaatggcgccgcgtgagtaaggccccggaggccctcttctttgttcagttcgagaagggcgagtcctacttccacctccatattctggtagagaccacgggggtcaaatccatggtgctgggccgcttcctgagtcagattcgggacaagctggtgcagaccatctaccgcgggatcgagccgaccctgcccaactggttcgcggtgacaaagacgcgtaatggcgccggaggggggaacaaggtggtggacgagtgctacatccccaactacctgctgcccaagactcagcccgagctgcagtgggcgtggactaacatggaggagtatataagcgcgtgcttgaacctggccgagcgcaaacggctcgtggcgcagcacctgacccacgtcagccagacccaggagcagaacaaggagaatctgaacccgaattctgacgcgcctgtcatccggtcaaaaacctccgcgcgctacatggagctggtcgggtggctggtggaccggggcatcacctccgagaagcagtggatccaggaggaccaggcctcgtacatctccttcaacgccgcctccaactcgcggtctcagatcaaggccgcgctggacaatgccggcaagatcatggcgctgaccaaatccgcgcccgactacctggtaggccccgctctgcccgcggacattaaatccaaccgcatctaccgcatcctggagctgaatggctacgaccctgcctacgccggttccgtctttctcggctgggcccagaaaaagtttggcaaaaggaacaccatctggctgtttgggccggccaccacgggcaagaccaacatcgcggaagccatcgcccacgccgtgcccttctacggctgcgtcaactggaccaatgagaactttcccttcaacgattgcgtcgacaagatggtgatctggtgggaggagggcaagatgacggccaaggtcgtggagtccgccaaggccattctcggcggcagcaaggtgcgcgtggaccaaaagtgcaagtcgtccgcccagatcgatcccacccccgtgatcgtcacctccaacaccaacatgtgcgccgtgattgacgggaacagcaccaccttcgagcaccagcagccgttgcaggaccggatgttcaaatttgaacttacccgccgtctggagcacgactttggcaaggtgacaaagcaggaagtcaaagagttcttccgctgggcgcaggatcacgtgaccgaggtggcgcatgagttctacgtcagaaagggtggagctaacaaaagacccgcccccgatgacgcggatataagcgagcccaagcgggcctgcccctcagtcgcggatccatcgacgtcagacgcggaaggagctccggtggactttgccgacaggtaccaaaacaaatgttctcgtcacgcgggcatgcttcagatgctgtttccctgcaaaacatgcgagagaatgaatcagaatttcaacatttgcttcacgcacgggaccagagactgttcagaatgtttccctggcgtgtcagaatctcaaccggtcgtcagaaaaaagacgtatcggaaactctgtgcgattcatcatctgctggggcgggcacccgagattgcttgctcggcctgcgacctggtcaacgtggacctggatgactgtgtttctgagcaataaatgacttaaaccaggtatggctgccgatggttatcttccagattggctcgaggacaacctctctgagggcattcgcgagtggtgggacctgaaacctggagccccgaaacccaaagccaaccagcaaaagcaggacaacggccggggtctggtgcttcctggctacaagtacctcggacccttcaacggactcgacaagggggagcccgtcaacgcggcggacgcagcggccctcgagcacgacaaggcctacgaccagcagctccaagcgggtgacaatccgtacctgcggtataatcacgccgacgccgagtttcaggagcgtctgcaagaagatacgtcttttgggggcaacctcgggcgcgcagtcttccaggccaaaaagcgggttctcgaacctctgggcctggttgaatcgccggttaagacggctcctggaaagaagagaccggtagagccatcaccccagcgctctccagactcctctacgggcatcggcaagaaaggccagcagcccgcaaaaaagagactcaattttgggcagactggcgactcagagtcagtccccgaccctcaaccaatcggagaaccaccagcaggcccctctggtctgggatctggtacaatggctgcaggcggtggcgctccaatggcagacaataacgaaggcgccgacggagtgggtagttcctcaggaaattggcattgcgattccacatggctgggcgacagagtcatcaccaccagcacccgcacctgggccctgcccacctacaacaaccacctctacaagcaaatctccaacgggacctcgggaggaagcaccaacgacaacacctacttcggctacagcaccccctgggggtattttgacttcaacagattccactgccacttttcaccacgtgactggcagcgactcatcaacaacaactggggattccggcccaagaggctcaacttcaagctcttcaacatccaagtcaaggaggtcacgcagaatgaaggcaccaagaccatcgccaataaccttaccagcacgattcaggtctttacggactcggaataccagctcccgtacgtgctcggctcggcgcaccagggctgcctgcctccgttcccggcggacgtcttcatgattcctcagtacgggtacctgactctgaacaatggcagtcaggctgtgggccggtcgtccttctactgcctggagtactttccttctcaaatgctgagaacgggcaacaactttgaattcagctacaacttcgaggacgtgcccttccacagcagctacgcgcacagccagagcctggaccggctgatgaaccctctcatcgaccagtacttgtactacctgtcccggactcaaagcacgggcggtactgcaggaactcagcagttgctattttctcaggccgggcctaacaacatgtcggctcaggccaagaactggctacccggtccctgctaccggcagcaacgcgtctccacgacactgtcgcagaacaacaacagcaactttgcctggacgggtgccaccaagtatcatctgaatggcagagactctctggtgaatcctggcgttgccatggctacccacaaggacgacgaagagcgattttttccatccagcggagtcttaatgtttgggaaacagggagctggaaaagacaacgtggactatagcagcgtgatgctaaccagcgaggaagaaataaagaccaccaacccagtggccacagaacagtacggcgtggtggccgataacctgcaacagcaaaacgccgctcctattgtaggggccgtcaatagtcaaggagccttacctggcatggtgtggcagaaccgggacgtgtacctgcagggtcccatctgggccaagattcctcatacggacggcaactttcatccctcgccgctgatgggaggctttggactgaagcatccgcctcctcagatcctgattaaaaacacacctgttcccgcggatcctccgaccaccttcactaaggccaagctggcttctttcatcacgcagtacagtaccggccaggtcagcgtggagatcgagtgggagctgcagaaggagaacagcaaacgctggaacccagagattcagtacacttccaactactacaaatctacaaatgtggactttgctgtcaatactgagggtacttattccgagcctcgccccattggcacccgttacctcacccgtaatctgtaattacatgttaatcaataaaccggttaattcgtttcagttgaactttggtctcctgtccttcttatcttatcggttaccatagaaactggttacttattaactgcttggtgcgcttcgcgataaaagacttacgtcatcgggttacccctagtgatgga

SEQ ID NO: 15 - DNA, 2052 bp, Adeno-associated virus
cgaccgcgcgagcgagcgagtgactccggcgggcccgtttcgggcccgcagcccgctggaaaccagcgggccggagtcactcgctcgctcgcgcgtctctccctcaccggttgaggtagtgatccccaaggaacatcaattactaattgggcggtacgatgaatagatgcatcggtacgagatctattgttgtatcctcgacactaaccgacaaaagtcggttagtcgtgactgagtaaacgtatcggaaatgttcgccagtgtttgagttctttgctcgccaaaattatcagaaaatcttataacaaatagcttggcttattccttgacacgaaacactaagtgtatagtcacctccccacacctttaccgtggaactagagtgggagtagctttcacctcaactacaggaagggaccgagcgatgtctgcgtgaaggcgttcaaaagaaaacttctagaagagaaagtagatttaaaaacctcgtccaaaagactgaagccagccttttggggagggttaaagtgaccagatgttactttcgttttgtcaagagaaggggcgaggggccacacactctccccgaaactaggaagagaccaaaggatcctttgcgcatacaccgatctattgttgtatcctcgacactaaccgacaaaagtcggttagtcgtgactgagtaaacgtatcggaaatgttcgccagtgtttgagttctttgctcgccaaaattatcagaaaatcttataacaaatagcttggcttattccttgacacgaaacactaagtgtatagtcacctccccacacctttaccgtggaactagagtgggagtagctttcacctcaactacaggaagggaccgagcgatgtctgcgtgaaggcgtttaagaatggaatcttttaacacgttaaaaacctcgtccaaaagactgaagccagccttttggggagggttaaagtgaccagatgttactttcgttttgtcaagagaaggggcgaggggccacacactctccccgaaactaggaagagaccaaaggatcctttgcgcatacaccgatctattgttgtatcctcgacactaaccgacaaaagtcggttagtcgtgactgagtaaacgtatcggaaatgttcgccagtgtttgagttctttgctcgccaaaattatcagaaaatcttataacaaatagcttggcttattccttgacacgaaacactaagtgtatagtcacctccccacacctttaccgtggaactagagtgggagtagctttcacctcaactacaggaagggaccgagcgatgtctgcgtgaaggcgtttaagaatggaatcttttaacacgttaaaaacctcgtccaaaagactgaagccagccttttggggagggttaaagtgaccagatgttactttcgttttgtcaagagaaggggcgaggggccacacactctccccgaaactaggaagagaccaaaggatcctttgcgcatacaccgatctattgttgtatcctcgacactaaccgacaaaagtcggttagtcgtgactgagtaaacgtatcggaaatgttcgccagtgtttgagttctttgctcgccaaaattatcagaaaatcttataacaaatagcttggcttattccttgacacgaaacactaagtgtatagtcacctccccacacctttaccgtggaactagagtgggagtagctttcacctcaactacaggaagggaccgagcgatgtctgcgtgaaggcgttcaaaagaaaacttctagaagagaaagtagatttaaaaacctcgtccaaaagactgaagccagccttttggggagggttaaagtgaccagatgttactttcgttttgtcaagagaaggggcgaggggccacacactctccccgaaactaggaagagaccaaaggatcctttgcgcatacacatgttggggtgagggagagacgcgcgagcgagcgagtgactccggcccgctggtttccagcgggctgcgggcccgaaacgggcccgccggagtcactcgctcgctcgcgcgtc

SEQ ID NO: 16 - protein, 8 aa, Homo sapiens
WVNAQFSK

SEQ ID NO: 17 - protein, 14 aa, Homo sapiens
QHIENLFSDLQDGR

SEQ ID NO: 18 - protein, 12 aa, Homo sapiens
LLDLLEGLTGQK

SEQ ID NO: 19 - protein, 23 aa, Homo sapiens
VLQNNNVDLVNIGSTDIVDGNHK

SEQ ID NO: 20 - protein, 13 aa, Homo sapiens
NLMAGLQQTNSEK

SEQ ID NO: 21 - protein, 9 aa, Homo sapiens
LEHAFNIAR

SEQ ID NO: 22 - protein, 7 aa, Homo sapiens
YQLGIEK

SEQ ID NO: 23 - protein, 15 aa, Homo sapiens
LLDPEDVDTTYPDKK

SEQ ID NO: 24 - protein, 17 aa, Homo sapiens
SYAYTQAAYVTTSDPTR

SEQ ID NO: 25 - protein, 14 aa, Homo sapiens
SPFPSQHLEAPEDK

SEQ ID NO: 26 - DNA, 2052 bp, Adeno-associated virus
gctggcgcgctcgctcgctcactgaggccgcccgggcaaagcccgggcgtcgggcgacctttggtcgcccggcctcagtgagcgagcgagcgcgcagagagggagtggccaactccatcactaggggttccttgtagttaatgattaacccgccatgctacttatctacgtagccatgctctagataacaacataggagctgtgattggctgttttcagccaatcagcactgactcatttgcatagcctttacaagcggtcacaaactcaagaaacgagcggttttaatagtcttttagaatattgtttatcgaaccgaataaggaactgtgctttgtgattcacatatcagtggaggggtgtggaaatggcaccttgatctcaccctcatcgaaagtggagttgatgtccttccctggctcgctacagacgcacttccgcaagttttcttttgaagatcttctctttcatctaaatttttggagcaggttttctgacttcggtcggaaaacccctcccaatttcactggtctacaatgaaagcaaaacagttctcttccccgctccccggtgtgtgagaggggctttgatccttctctggtttcctaggaaacgcgtatgtggctagataacaacataggagctgtgattggctgttttcagccaatcagcactgactcatttgcatagcctttacaagcggtcacaaactcaagaaacgagcggttttaatagtcttttagaatattgtttatcgaaccgaataaggaactgtgctttgtgattcacatatcagtggaggggtgtggaaatggcaccttgatctcaccctcatcgaaagtggagttgatgtccttccctggctcgctacagacgcacttccgcaaattcttaccttagaaaattgtgcaatttttggagcaggttttctgacttcggtcggaaaacccctcccaatttcactggtctacaatgaaagcaaaacagttctcttccccgctccccggtgtgtgagaggggctttgatccttctctggtttcctaggaaacgcgtatgtggctagataacaacataggagctgtgattggctgttttcagccaatcagcactgactcatttgcatagcctttacaagcggtcacaaactcaagaaacgagcggttttaatagtcttttagaatattgtttatcgaaccgaataaggaactgtgctttgtgattcacatatcagtggaggggtgtggaaatggcaccttgatctcaccctcatcgaaagtggagttgatgtccttccctggctcgctacagacgcacttccgcaaattcttaccttagaaaattgtgcaatttttggagcaggttttctgacttcggtcggaaaacccctcccaatttcactggtctacaatgaaagcaaaacagttctcttccccgctccccggtgtgtgagaggggctttgatccttctctggtttcctaggaaacgcgtatgtggctagataacaacataggagctgtgattggctgttttcagccaatcagcactgactcatttgcatagcctttacaagcggtcacaaactcaagaaacgagcggttttaatagtcttttagaatattgtttatcgaaccgaataaggaactgtgctttgtgattcacatatcagtggaggggtgtggaaatggcaccttgatctcaccctcatcgaaagtggagttgatgtccttccctggctcgctacagacgcacttccgcaagttttcttttgaagatcttctctttcatctaaatttttggagcaggttttctgacttcggtcggaaaacccctcccaatttcactggtctacaatgaaagcaaaacagttctcttccccgctccccggtgtgtgagaggggctttgatccttctctggtttcctaggaaacgcgtatgtgtacaaccccactccctctctgcgcgctcgctcgctcactgaggccgggcgaccaaaggtcgcccgacgcccgggctttgcccgggcggcctcagtgagcgagcgagcgcgcag

SEQ ID NO: 27 - protein, 240 aa, Homo sapiens
  ref <308>: UniProtKB/Swiss-Prot: P11532.3
  ref <309>: 2015-07-22
  ref <313>: (1)..(240)
MLWWEEVEDCYEREDVQKKTFTKWVNAQFSKFGKQHIENLFSDLQDGRRLLDLLEGLTGQKLPKEKGSTRVHALNNVNKALRVLQNNNVDLVNIGSTDIVDGNHKLTLGLIWNIILHWQVKNVMKNIMAGLQQTNSEKILLSWVRQSTRNYPQVNVINFTTSWSDGLALNALIHSHRPDLFDWNSVVCQQSATQRLEHAFNIARYQLGIEKLLDPEDVDTTYPDKKSILMYITSLFQVLP

SEQ ID NO: 28 - protein, 22 aa, Homo sapiens
YQLGIEKLLDPEDVDTTYPDKK

SEQ ID NO: 29 - protein, 122 aa, Homo sapiens
WVNAQFSKFGKQHIENLFSDLQDGRRLLDLLEGLTGQKVLQNNNVDLVNIGSTDIVDGNHKNIMAGLQQTNSEKILLLEHAFNIARYQLGIEKLLDPEDVDTTYPDKKSILMYITSLFQVLP

SEQ ID NO: 30 - DNA, 75 bp, Homo sapiens
tagatgaaagagaagatgttcaaaagaaaacattcacaaaatgggtaaatgcacaattttctaaggtaagaatgg

SEQ ID NO: 31 - DNA, 80 bp, Homo sapiens
aactccatttatcaattaaccaaaaactcccaaataactgtgtaggttccatgagttcaggagattccacttcaactaat

SEQ ID NO: 32 - DNA, 80 bp, Homo sapiens
aactccatttatcaattaaccaaaaactcccaaataactgtggtgtatatttatctatttttatgggttgcaaaatactt

SEQ ID NO: 33 - DNA, 80 bp, Homo sapiens
caaattctcccctgaaaatttaaaaaaatacattgttctgtggtgtatatttatctatttttatgggttgcaaaatactt

SEQ ID NO: 34 - DNA, 55 bp, Homo sapiens
aattaaccaaaaactcccaaataactgtggtgtatatttatctatttttatgggt